European Patent Specification EP 3 211 420 B1, published July 24, 2024. Title: Assay for Detection of Chimeric Antigen Receptor T cells. Applicant: Miltenyi Biotec GmbH. Application EP2016157802.6. The sequence listing filed with the application follows.

SEQUENCE LISTING (3 sequences)

SEQ ID NO: 1 - protein, 17 aa, Homo sapiens
CEPANPSEKNSPSTQYC

SEQ ID NO: 2 - protein, 25 aa, Homo sapiens [sequence omitted]

SEQ ID NO: 3 - protein, 5 aa, Homo sapiens
GGGSK